European Patent Application EP 4 722 254 A1, published April 8, 2026. Title: 一种抗FGFR2/PD-1双特异性抗体. Applicant: 三生国健药业（上海）股份有限公司. The sequence listing filed with the application follows.

SEQUENCE LISTING (33 sequences)

SEQ ID NO: 1 - protein, 5 aa, synthetic construct
  source 1..5: note = Amino acid sequence of HCDR1 of anti-FGFR2 monoclonal antibody
SYWMH

SEQ ID NO: 2 - protein, 17 aa, synthetic construct
  source 1..17: note = Amino acid sequence of HCDR2 of anti-FGFR2 monoclonal antibody
AIYPGNSDTDYSGKFKG

SEQ ID NO: 3 - skipped

SEQ ID NO: 4 - protein, 12 aa, synthetic construct
  source 1..12: note = Amino acid sequence of LCDR1 of anti-FGFR2 monoclonal antibody
RASSSVNYMYWY

SEQ ID NO: 5 - protein, 7 aa, synthetic construct
  source 1..7: note = Amino acid sequence of LCDR2 of anti-FGFR2 monoclonal antibody
LTSNRAT

SEQ ID NO: 6 - protein, 9 aa, synthetic construct
  source 1..9: note = Amino acid sequence of LCDR3 of anti-FGFR2 monoclonal antibody
QQWSSNPYT

SEQ ID NO: 7 - protein, 5 aa, synthetic construct
  source 1..5: note = Amino acid sequence of HCDR1 of anti-PD-1 monoclonal antibody
SYDMS

SEQ ID NO: 8 - protein, 17 aa, synthetic construct
  source 1..17: note = Amino acid sequence of HCDR2 of anti-PD-1 monoclonal antibody
TISGGGRYTYYPDTVKG

SEQ ID NO: 9 - protein, 8 aa, synthetic construct
  source 1..8: note = Amino acid sequence of HCDR3 of anti-PD-1 monoclonal antibody
PYGGYFDV

SEQ ID NO: 10 - protein, 11 aa, synthetic construct
  source 1..11: note = Amino acid sequence of LCDR1 of anti-PD-1 monoclonal antibody
RASQSISNFLH

SEQ ID NO: 11 - protein, 7 aa, synthetic construct
  source 1..7: note = Amino acid sequence of LCDR2 of anti-PD-1 monoclonal antibody
YASQSIS

SEQ ID NO: 12 - protein, 9 aa, synthetic construct
  source 1..9: note = Amino acid sequence of LCDR3 of anti-PD-1 monoclonal antibody
QQSNSWPHT

SEQ ID NO: 13 - protein, 112 aa, synthetic construct
  source 1..112: note = amino acid sequence of VH of anti-FGFR2 monoclonal antibody
QVQLVQSGAEVKKPGSSVKVSCKASGYTFTSYWMHWVRQAPGQGLEWMGAIYPGNSDTDYSGKFKGRVTITADESTSTAYMELSSLRSEDTAVYYCSKFDYWGQGTLVTVSS

SEQ ID NO: 14 - protein, 109 aa, synthetic construct
  source 1..109: note = amino acid sequence of VL of anti-FGFR2 monoclonal antibody
EIVLTQSPATLSLSPGERATLSCRASSSVNYMYWYQQKPGQAPRPWIYLTSNRATGVPARFSGSGSGTDYTLTISSLEPEDFAVYYCQQWSSNPYTFGQGTKLEIKRTV

SEQ ID NO: 15 - protein, 117 aa, synthetic construct
  source 1..117: note = amino acid sequence of VH of anti-PD-1 monoclonal antibody
EVKLVESGGGLVQPGGSLRLSCAASGFAFSSYDMSWVRQAPGKRLEWVATISGGGRYTYYPDTVKGRFTISRDNAKNSHYLQMNSLRAEDTAVYFCASPYGGYFDVWGQGTLVTVSS

SEQ ID NO: 16 - protein, 107 aa, synthetic construct
  source 1..107: note = amino acid sequence of VL of anti-PD-1 monoclonal antibody
EIVLTQSPATLSLSPGERATLSCRASQSISNFLHWYQQKPGQAPRLLIKYASQSISGIPARFSGSGSGTDFTLTISSLEPEDFAVYFCQQSNSWPHTFGQGTKVEIK

SEQ ID NO: 17 - protein, 20 aa, synthetic construct
  source 1..20: note = Amino acid sequence of peptide linker L1
GGGGSGGGGSGGGGSGGGGS

SEQ ID NO: 18 - protein, 15 aa, synthetic construct
  source 1..15: note = Amino acid sequence of peptide linker L2
GGGGSGGGGSGGGGS

SEQ ID NO: 19 - protein, 98 aa, synthetic construct
  source 1..98: note = amino acid sequence of heavy chain constant CH1
ASTKGPSVFPLAPSSKSTSGGTAALGCLVKDYFPEPVTVSWNSGALTSGVHTFPAVLQSSGLYSLSSVVTVPSSSLGTQTYICNVNHKPSNTKVDKKV

SEQ ID NO: 20 - protein, 109 aa, synthetic construct
  source 1..109: note = amino acid sequence of heavy chain constant CH2
PAPELLGGPSVFLFPPKPKDTLMISRTPEVTCVVVDVSHEDPEVKFNWYVDGVEVHNAKTKPREEQYNSTYRVVSVLTVLHQDWLNGKEYKCKVSNKALPAPIEKTISK

SEQ ID NO: 21 - protein, 109 aa, synthetic construct
  source 1..109: note = amino acid sequence of heavy chain constant CH3
AKGQPREPQVYTLPPSREEMTKNQVSLTCLVKGFYPSDIAVEWESNGQPENNYKTTPPVLDSDGSFFLYSKLTVDKSRWQQGNVFSCSVMHEALHNHYTQKSLSLSPGK

SEQ ID NO: 22 - protein, 109 aa, synthetic construct
  source 1..109: note = amino acid sequence of heavy chain constant region CH2-S239D-I332E
PAPELLGGPDVFLFPPKPKDTLMISRTPEVTCVVVDVSHEDPEVKFNWYVDGVEVHNAKTKPREEQYNSTYRVVSVLTVLHQDWLNGKEYKCKVSNKALPAPEEKTISK

SEQ ID NO: 23 - protein, 330 aa, synthetic construct
  source 1..330: note = amino acid sequence of heavy chain constant CH
ASTKGPSVFPLAPSSKSTSGGTAALGCLVKDYFPEPVTVSWNSGALTSGVHTFPAVLQSSGLYSLSSVVTVPSSSLGTQTYICNVNHKPSNTKVDKKVEPKSCDKTHTCPPCPAPELLGGPSVFLFPPKPKDTLMISRTPEVTCVVVDVSHEDPEVKFNWYVDGVEVHNAKTKPREEQYNSTYRVVSVLTVLHQDWLNGKEYKCKVSNKALPAPIEKTISKAKGQPREPQVYTLPPSREEMTKNQVSLTCLVKGFYPSDIAVEWESNGQPENNYKTTPPVLDSDGSFFLYSKLTVDKSRWQQGNVFSCSVMHEALHNHYTQKSLSLSPGK

SEQ ID NO: 24 - protein, 330 aa, synthetic construct
  source 1..330: note = amino acid sequence of heavy chain constant region CH-S239D-I332E
ASTKGPSVFPLAPSSKSTSGGTAALGCLVKDYFPEPVTVSWNSGALTSGVHTFPAVLQSSGLYSLSSVVTVPSSSLGTQTYICNVNHKPSNTKVDKKVEPKSCDKTHTCPPCPAPELLGGPDVFLFPPKPKDTLMISRTPEVTCVVVDVSHEDPEVKFNWYVDGVEVHNAKTKPREEQYNSTYRVVSVLTVLHQDWLNGKEYKCKVSNKALPAPEEKTISKAKGQPREPQVYTLPPSREEMTKNQVSLTCLVKGFYPSDIAVEWESNGQPENNYKTTPPVLDSDGSFFLYSKLTVDKSRWQQGNVFSCSVMHEALHNHYTQKSLSLSPGK

SEQ ID NO: 25 - protein, 442 aa, synthetic construct
  source 1..442: note = amino acid sequence of heavy chain of anti-FGFR2 monoclonal antibody
QVQLVQSGAEVKKPGSSVKVSCKASGYTFTSYWMHWVRQAPGQGLEWMGAIYPGNSDTDYSGKFKGRVTITADESTSTAYMELSSLRSEDTAVYYCSKFDYWGQGTLVTVSSASTKGPSVFPLAPSSKSTSGGTAALGCLVKDYFPEPVTVSWNSGALTSGVHTFPAVLQSSGLYSLSSVVTVPSSSLGTQTYICNVNHKPSNTKVDKKVEPKSCDKTHTCPPCPAPELLGGPSVFLFPPKPKDTLMISRTPEVTCVVVDVSHEDPEVKFNWYVDGVEVHNAKTKPREEQYNSTYRVVSVLTVLHQDWLNGKEYKCKVSNKALPAPIEKTISKAKGQPREPQVYTLPPSREEMTKNQVSLTCLVKGFYPSDIAVEWESNGQPENNYKTTPPVLDSDGSFFLYSKLTVDKSRWQQGNVFSCSVMHEALHNHYTQKSLSLSPGK

SEQ ID NO: 26 - protein, 442 aa, synthetic construct
  source 1..442: note = amino acid sequence of heavy chain HC-S239D-I332E of anti-FGFR2 monoclonal antibody
QVQLVQSGAEVKKPGSSVKVSCKASGYTFTSYWMHWVRQAPGQGLEWMGAIYPGNSDTDYSGKFKGRVTITADESTSTAYMELSSLRSEDTAVYYCSKFDYWGQGTLVTVSSASTKGPSVFPLAPSSKSTSGGTAALGCLVKDYFPEPVTVSWNSGALTSGVHTFPAVLQSSGLYSLSSVVTVPSSSLGTQTYICNVNHKPSNTKVDKKVEPKSCDKTHTCPPCPAPELLGGPDVFLFPPKPKDTLMISRTPEVTCVVVDVSHEDPEVKFNWYVDGVEVHNAKTKPREEQYNSTYRVVSVLTVLHQDWLNGKEYKCKVSNKALPAPEEKTISKAKGQPREPQVYTLPPSREEMTKNQVSLTCLVKGFYPSDIAVEWESNGQPENNYKTTPPVLDSDGSFFLYSKLTVDKSRWQQGNVFSCSVMHEALHNHYTQKSLSLSPGK

SEQ ID NO: 27 - protein, 244 aa, synthetic construct
  source 1..244: note = amino acid sequence of scFv-VLVH of anti-PD-1 monoclonal antibody
EIVLTQSPATLSLSPGERATLSCRASQSISNFLHWYQQKPGQAPRLLIKYASQSISGIPARFSGSGSGTDFTLTISSLEPEDFAVYFCQQSNSWPHTFGQGTKVEIKGGGGSGGGGSGGGGSGGGGSEVKLVESGGGLVQPGGSLRLSCAASGFAFSSYDMSWVRQAPGKRLEWVATISGGGRYTYYPDTVKGRFTISRDNAKNSHYLQMNSLRAEDTAVYFCASPYGGYFDVWGQGTLVTVSS

SEQ ID NO: 28 - protein, 213 aa, synthetic construct
  source 1..213: note = amino acid sequence of light chain of anti-FGFR2/PD-1 double antibody a/b
EIVLTQSPATLSLSPGERATLSCRASSSVNYMYWYQQKPGQAPRPWIYLTSNRATGVPARFSGSGSGTDYTLTISSLEPEDFAVYYCQQWSSNPYTFGQGTKLEIKRTVAAPSVFIFPPSDEQLKSGTASVVCLLNNFYPREAKVQWKVDNALQSGNSQESVTEQDSKDSTYSLSSTLTLSKADYEKHKVYACEVTHQGLSSPVTKSFNRGEC

SEQ ID NO: 29 - protein, 701 aa, synthetic construct
  source 1..701: note = amino acid sequence of heavy chain of anti-FGFR2/PD-1 double antibody a
QVQLVQSGAEVKKPGSSVKVSCKASGYTFTSYWMHWVRQAPGQGLEWMGAIYPGNSDTDYSGKFKGRVTITADESTSTAYMELSSLRSEDTAVYYCSKFDYWGQGTLVTVSSASTKGPSVFPLAPSSKSTSGGTAALGCLVKDYFPEPVTVSWNSGALTSGVHTFPAVLQSSGLYSLSSVVTVPSSSLGTQTYICNVNHKPSNTKVDKKVEPKSCDKTHTCPPCPAPELLGGPSVFLFPPKPKDTLMISRTPEVTCVVVDVSHEDPEVKFNWYVDGVEVHNAKTKPREEQYNSTYRVVSVLTVLHQDWLNGKEYKCKVSNKALPAPIEKTISKAKGQPREPQVYTLPPSREEMTKNQVSLTCLVKGFYPSDIAVEWESNGQPENNYKTTPPVLDSDGSFFLYSKLTVDKSRWQQGNVFSCSVMHEALHNHYTQKSLSLSPGKGGGGSGGGGSGGGGSEIVLTQSPATLSLSPGERATLSCRASQSISNFLHWYQQKPGQAPRLLIKYASQSISGIPARFSGSGSGTDFTLTISSLEPEDFAVYFCQQSNSWPHTFGQGTKVEIKGGGGSGGGGSGGGGSGGGGSEVKLVESGGGLVQPGGSLRLSCAASGFAFSSYDMSWVRQAPGKRLEWVATISGGGRYTYYPDTVKGRFTISRDNAKNSHYLQMNSLRAEDTAVYFCASPYGGYFDVWGQGTLVTVSS

SEQ ID NO: 30 - protein, 701 aa, synthetic construct
  source 1..701: note = amino acid sequence of heavy chain of anti-FGFR2/PD-1 double antibody b
QVQLVQSGAEVKKPGSSVKVSCKASGYTFTSYWMHWVRQAPGQGLEWMGAIYPGNSDTDYSGKFKGRVTITADESTSTAYMELSSLRSEDTAVYYCSKFDYWGQGTLVTVSSASTKGPSVFPLAPSSKSTSGGTAALGCLVKDYFPEPVTVSWNSGALTSGVHTFPAVLQSSGLYSLSSVVTVPSSSLGTQTYICNVNHKPSNTKVDKKVEPKSCDKTHTCPPCPAPELLGGPDVFLFPPKPKDTLMISRTPEVTCVVVDVSHEDPEVKFNWYVDGVEVHNAKTKPREEQYNSTYRVVSVLTVLHQDWLNGKEYKCKVSNKALPAPEEKTISKAKGQPREPQVYTLPPSREEMTKNQVSLTCLVKGFYPSDIAVEWESNGQPENNYKTTPPVLDSDGSFFLYSKLTVDKSRWQQGNVFSCSVMHEALHNHYTQKSLSLSPGKGGGGSGGGGSGGGGSEIVLTQSPATLSLSPGERATLSCRASQSISNFLHWYQQKPGQAPRLLIKYASQSISGIPARFSGSGSGTDFTLTISSLEPEDFAVYFCQQSNSWPHTFGQGTKVEIKGGGGSGGGGSGGGGSGGGGSEVKLVESGGGLVQPGGSLRLSCAASGFAFSSYDMSWVRQAPGKRLEWVATISGGGRYTYYPDTVKGRFTISRDNAKNSHYLQMNSLRAEDTAVYFCASPYGGYFDVWGQGTLVTVSS

SEQ ID NO: 31 - DNA, 2103 bp, synthetic construct
  source 1..2103: mol_type = other DNA; note = nucleotide sequence of heavy chain of anti-FGFR2/PD-1 double antibody a
caggtgcagctggtgcagtccggcgccgaggtgaagaagcctggctccagcgtgaaggtgtcttgcaaggccagcggctacaccttcacctcctactggatgcactgggtgaggcaggcccccggccagggcctggagtggatgggcgccatctaccctggcaacagcgacaccgactattccggcaagttcaagggccgggtgaccatcaccgccgacgagtccacctccaccgcctacatggagctgagcagcctgaggtccgaggacaccgccgtgtactactgcagcaagttcgactactggggccagggcaccctggtgaccgtgtcctccgcgagcaccaagggaccttccgtgtttcccctcgcccccagctccaaaagcaccagcggcggaacagctgctctcggctgtctcgtcaaggattacttccccgagcccgtgaccgtgagctggaacagcggagccctgacaagcggcgtccacaccttccctgctgtcctacagtcctccggactgtacagcctgagcagcgtggtgacagtccctagcagctccctgggcacccagacatatatttgcaacgtgaatcacaagcccagcaacaccaaggtcgataagaaggtggagcctaagtcctgcgacaagacccacacatgtcccccctgtcccgctcctgaactgctgggaggcccttccgtgttcctgttcccccctaagcccaaggacaccctgatgatttccaggacacccgaggtgacctgtgtggtggtggacgtcagccacgaggaccccgaggtgaaattcaactggtacgtcgatggcgtggaggtgcacaacgctaagaccaagcccagggaggagcagtacaattccacctacagggtggtgtccgtgctgaccgtcctccatcaggactggctgaacggcaaagagtataagtgcaaggtgagcaacaaggccctccctgctcccatcgagaagaccatcagcaaagccaagggccagcccagggaacctcaagtctataccctgcctcccagcagggaggagatgaccaagaaccaagtgagcctcacatgcctcgtcaagggcttctatccttccgatattgccgtcgagtgggagtccaacggacagcccgagaacaactacaagacaacaccccccgtgctcgattccgatggcagcttcttcctgtactccaagctgaccgtggacaagtccagatggcaacaaggcaacgtcttcagttgcagcgtcatgcatgaggccctccacaaccactacacccagaagagcctctccctgagccctggaaagggcggtgggggtagtggaggcggaggttcgggagggggcggtagcgagatcgtccttacccaatcaccagcaaccttgtcactgtcaccaggtgaaagagcaaccctcagttgtagggctagtcagagtatctccaacttcctgcactggtaccagcagaagcctggacaggcccctcggttgctcattaagtacgcctctcaatctatcagcggaatccccgctcgcttttctggctctggctccgggactgatttcactctgacaatttccagcctggaacccgaggactttgccgtttatttttgccagcagagcaatagctggccccatacattcgggcagggcacaaaagtggagataaaaggtggaggcggttcaggcggaggtggcagcggcggtggcgggtcgggagggggtggctctgaagtcaaactcgtggagtccggcggaggcctcgttcaaccaggtggatctcttcgtttgtcctgcgcagcatcaggattcgctttctccagctacgacatgagctgggtccgacaggctcctggaaagaggctggaatgggttgctactatcagcggcggtggtagatatacttattaccccgataccgtaaaggggaggttcaccattagtcgcgataacgccaaaaattcacactacctgcagatgaactctctgcgggccgaggacaccgccgtgtacttttgtgccagtccctatggcgggtattttgacgtgtggggccaggggacactggtgactgtgagttct

SEQ ID NO: 32 - DNA, 2103 bp, synthetic construct
  source 1..2103: mol_type = other DNA; note = nucleotide sequence of heavy chain of anti-FGFR2/PD-1 double antibody b
caggtgcagctggtgcagtccggcgccgaggtgaagaagcctggctccagcgtgaaggtgtcttgcaaggccagcggctacaccttcacctcctactggatgcactgggtgaggcaggcccccggccagggcctggagtggatgggcgccatctaccctggcaacagcgacaccgactattccggcaagttcaagggccgggtgaccatcaccgccgacgagtccacctccaccgcctacatggagctgagcagcctgaggtccgaggacaccgccgtgtactactgcagcaagttcgactactggggccagggcaccctggtgaccgtgtcctccgcgagcaccaagggaccttccgtgtttcccctcgcccccagctccaaaagcaccagcggcggaacagctgctctcggctgtctcgtcaaggattacttccccgagcccgtgaccgtgagctggaacagcggagccctgacaagcggcgtccacaccttccctgctgtcctacagtcctccggactgtacagcctgagcagcgtggtgacagtccctagcagctccctgggcacccagacatatatttgcaacgtgaatcacaagcccagcaacaccaaggtcgataagaaggtggagcctaagtcctgcgacaagacccacacatgtcccccctgtcccgctcctgaactgctgggaggccctgacgtgttcctgttcccccctaagcccaaggacaccctgatgatttccaggacacccgaggtgacctgtgtggtggtggacgtcagccacgaggaccccgaggtgaaattcaactggtacgtcgatggcgtggaggtgcacaacgctaagaccaagcccagggaggagcagtacaattccacctacagggtggtgtccgtgctgaccgtcctccatcaggactggctgaacggcaaagagtataagtgcaaggtgagcaacaaggccctccctgctcccgaggagaagaccatcagcaaagccaagggccagcccagggaacctcaagtctataccctgcctcccagcagggaggagatgaccaagaaccaagtgagcctcacatgcctcgtcaagggcttctatccttccgatattgccgtcgagtgggagtccaacggacagcccgagaacaactacaagacaacaccccccgtgctcgattccgatggcagcttcttcctgtactccaagctgaccgtggacaagtccagatggcaacaaggcaacgtcttcagttgcagcgtcatgcatgaggccctccacaaccactacacccagaagagcctctccctgagccctggaaagggcggtgggggtagtggaggcggaggttcgggagggggcggtagcgagatcgtccttacccaatcaccagcaaccttgtcactgtcaccaggtgaaagagcaaccctcagttgtagggctagtcagagtatctccaacttcctgcactggtaccagcagaagcctggacaggcccctcggttgctcattaagtacgcctctcaatctatcagcggaatccccgctcgcttttctggctctggctccgggactgatttcactctgacaatttccagcctggaacccgaggactttgccgtttatttttgccagcagagcaatagctggccccatacattcgggcagggcacaaaagtggagataaaaggtggaggcggttcaggcggaggtggcagcggcggtggcgggtcgggagggggtggctctgaagtcaaactcgtggagtccggcggaggcctcgttcaaccaggtggatctcttcgtttgtcctgcgcagcatcaggattcgctttctccagctacgacatgagctgggtccgacaggctcctggaaagaggctggaatgggttgctactatcagcggcggtggtagatatacttattaccccgataccgtaaaggggaggttcaccattagtcgcgataacgccaaaaattcacactacctgcagatgaactctctgcgggccgaggacaccgccgtgtacttttgtgccagtccctatggcgggtattttgacgtgtggggccaggggacactggtgactgtgagttct

SEQ ID NO: 33 - DNA, 639 bp, synthetic construct
  source 1..639: mol_type = other DNA; note = nucleotide sequence of light chain of anti-FGFR2/PD-1 double antibody a/b
gagatcgtgctgacccagtcccctgccaccctgtccctgtcccccggcgagcgggccaccctgtcttgccgggctagctcctccgtgaactacatgtactggtaccagcagaagcctggccaggcccctaggccctggatctacctgaccagcaacagggccaccggcgtgcccgccaggttctccggcagcggctccggcaccgactacaccctgaccatctcctccctggagcccgaggacttcgccgtgtactactgccagcagtggtctagcaatccctacactttcggccagggcaccaagctggagatcaagaggaccgtggccgccccctccgtgttcatttttccccctagcgacgagcagctgaagagcggcaccgctagcgtggtgtgcctgctgaacaacttctaccccagggaggccaaggtgcagtggaaagtggacaacgccctgcagagcggcaactcccaggagtccgtgaccgagcaggacagcaaggacagcacctactccctgtcctccaccctgaccctgtccaaggccgactacgagaagcacaaggtgtacgcctgtgaggtgacacaccagggcctgtcctcccccgtgacaaagtccttcaacaggggcgagtgc